European Patent Application EP 4 567 047 A1, published June 11, 2025. Title: RECOMBINANT ANTIBODY, KIT COMPRISING THE SAME, AND USES THEREOF IN DIAGNOSING CANCERS. Applicant: UNI PHARMA CO., LTD. The sequence listing filed with the application follows.

SEQUENCE LISTING (24 sequences)

SEQ ID NO: 1 - protein, 10 aa, synthetic construct
SGFAFNAYDM

SEQ ID NO: 2 - protein, 8 aa, synthetic construct
ISSSGDYT

SEQ ID NO: 3 - protein, 11 aa, synthetic construct
VYYHYDEGLDY

SEQ ID NO: 4 - protein, 148 aa, synthetic construct
MSTEHRHLTMNFGLRLIFLVLTLKGVKCEVQLVESGGGLVKPGGSLKLSCAASGFAFNAYDMSWVRQTPEKRLEWVAYISSSGDYTYYPDTVKGRFTVSRDNAKSTLYLHMGSLKSEDTAMYYCAVYYHYDEGLDYWGQGTALTVSSA

SEQ ID NO: 5 - protein, 9 aa, synthetic construct
ASSSVNYMH

SEQ ID NO: 6 - protein, 8 aa, synthetic construct
YDTSKLAS

SEQ ID NO: 7 - protein, 9 aa, synthetic construct
QQWSSNPPT

SEQ ID NO: 8 - protein, 129 aa, synthetic construct
MDFQVQIFSFLLISASVIISRGQIVLIQSPAIMSASPGEKVTMTCSASSSVNYMHWYQQKSGTSPKRWIYDTSKLASGVPARFSGSGSGTSYSLTISSMEAEDAATYYCQQWSSNPPTFGGGTKLEIKR

SEQ ID NO: 9 - protein, 24 aa, synthetic construct
EVQLVESGGGLVKPGGSLKLSCAA

SEQ ID NO: 10 - protein, 16 aa, synthetic construct
SWVRQTPEKRLEWVAY

SEQ ID NO: 11 - protein, 39 aa, synthetic construct
YYPDTVKGRFTVSRDNAKSTLYLHMGSLKSEDTAMYYCA

SEQ ID NO: 12 - protein, 12 aa, synthetic construct
WGQGTALTVSSA

SEQ ID NO: 13 - protein, 24 aa, synthetic construct
QIVLIQSPAIMSASPGEKVTMTCS

SEQ ID NO: 14 - protein, 14 aa, synthetic construct
WYQQKSGTSPKRWI

SEQ ID NO: 15 - protein, 32 aa, synthetic construct
GVPARFSGSGSGTSYSLTISSMEAEDAATYYC

SEQ ID NO: 16 - protein, 11 aa, synthetic construct
FGGGTKLEIKR

SEQ ID NO: 17 - protein, 10 aa, synthetic construct
GFTFSRSTMS

SEQ ID NO: 18 - protein, 9 aa, synthetic construct
TISSGGGFT

SEQ ID NO: 19 - protein, 12 aa, synthetic construct
TKYGSYVGYFDV

SEQ ID NO: 20 - protein, 148 aa, synthetic construct
MSSEHRPLTMNFGLRLIFLVLTLKGVQCDVKLVESGGGLVKPGGSLKLSCAASGFTFSRSTMSWVRQTPEKRLEWVATISSGGGFTYYPDTVRGRFTISRDNDKNTLYLQMSSLKSEDTAMYFCTKYGSYVGYFDVWGAGTTVTVSSA

SEQ ID NO: 21 - protein, 12 aa, synthetic construct
TASSSVSSSYLH

SEQ ID NO: 22 - protein, 7 aa, synthetic construct
STSNLSS

SEQ ID NO: 23 - protein, 9 aa, synthetic construct
HQYQRSPWT

SEQ ID NO: 24 - protein, 130 aa, synthetic construct
MDFQVQIFSFLLISASVIMSRGQIVLTQSPAIMSTSLGERVTMTCTASSSVSSSYLHWYQQKPGSSPKLWMYSTSNLSSGVPARFSGSGSGTSYSLTISSMEAEDAATYYCHQYQRSPWTFGGGTKLEIK